European Patent Application EP 4 733 315 A2, published April 29, 2026. Title: ANTAGONISTS AND AGONISTS OF THE TRANSFERRIN RECEPTOR-2 FOR USE IN THE TREATMENT OF DISEASES OF THE BONE. Applicant: Kymab Limited. Application EP. The sequence listing filed with the application follows.

SEQUENCE LISTING (114 sequences)

SEQ ID NO: 1 - protein, 697 aa, Homo Sapien
RGSCQACGDSVLVVSEDVNYEPDLDFHQGRLYWSDLQAMFLQFLGEGRLEDTIRQTSLRERVAGSAGMAALTQDIRAALSRQKLDHVWTDTHYVGLQFPDPAHPNTLHWVDEAGKVGEQLPLEDPDVYCPYSAIGNVTGELVYAHYGRPEDLQDLRARGVDPVGRLLLVRVGVISFAQKVTNAQDFGAQGVLIYPEPADFSQDPPKPSLSSQQAVYGHVHLGTGDPYTPGFPSFNQTQFPPVASSGLPSIPAQPISADIASRLLRKLKGPVAPQEWQGSLLGSPYHLGPGPRLRLVVNNHRTSTPINNIFGCIEGRSEPDHYVVIGAQRDAWGPGAAKSAVGTAILLELVRTFSSMVSNGFRPRRSLLFISWDGGDFGSVGSTEWLEGYLSVLHLKAVVYVSLDNAVLGDDKFHAKTSPLLTSLIESVLKQVDSPNHSGQTLYEQVVFTNPSWDAEVIRPLPMDSSAYSFTAFVGVPAVEFSFMEDDQAYPFLHTKEDTYENLHKVLQGRLPAVAQAVAQLAGQLLIRLSHDRLLPLDFGRYGDVVLRHIGNLNEFSGDLKARGLTLQWVYSARGDYIRAAEKLRQEIYSSEERDERLTRMYNVRIMRVEFYFLSQYVSPADSPFRHIFMGRGDHTLGALLDHLRLLRSNSSGTPGATSSTGFQESRFRRQLALLTWTLQGAANALSGDVWNIDNNF

SEQ ID NO: 2 - protein, 696 aa, Mus Musculus
RGSCQACGDSVLVVDEDVNPEDSGRTTLYWSDLQAMFLRFLGEGRMEDTIRLTSLRERVAGSARMATLVQDILDKLSRQKLDHVWTDTHYVGLQFPDPAHANTLHWVDADGSVQEQLPLEDPEVYCPYSATGNATGKLVYAHYGRSEDLQDLKAKGVELAGSLLLVRVGITSFAQKVAVAQDFGAQGVLIYPDPSDFSQDPHKPGLSSHQAVYGHVHLGTGDPYTPGFPSFNQTQFPPVESSGLPSIPAQPISADIADQLLRKLTGPVAPQEWKGHLSGSPYRLGPGPDLRLVVNNHRVSTPISNIFACIEGFAEPDHYVVIGAQRDAWGPGAAKSAVGTAILLELVRTFSSMVSNGFRPRRSLLFISWDGGDFGSVGATEWLEGYLSVLHLKAVVYVSLDNSVLGDGKFHAKTSPLLVSLIENILKQVDSPNHSGQTLYEQVALTHPSWDAEVIQPLPMDSSAYSFTAFAGVPAVEFSFMEDDRVYPFLHTKEDTYENLHKMLRGRLPAVVQAVAQLAGQLLIRLSHDHLLPLDFGRYGDVVLRHIGNLNEFSGDLKERGLTLQWVYSARGDYIRAAEKLRKEIYSSERNDERLMRMYNVRIMRVEFYFLSQYVSPADSPFRHIFLGQGDHTLGALVDHLRMLRADGSGAASSRLTAGLGFQESRFRRQLALLTWTLQGAANALSGDVWNIDNNF

SEQ ID NO: 3 - protein, 800 aa, Homo Sapien
MERLWGLFQRAQQLSPRSSQTVYQRVEGPRKGHLEEEEEDGEEGAETLAHFCPMELRGPEPLGSRPRQPNLIPWAAAGRRAAPYLVLTALLIFTGAFLLGYVAFRGSCQACGDSVLVVSEDVNYEPDLDFHQGRLYWSDLQAMFLQFLGEGRLEDTIRQTSLRERVAGSAGMAALTQDIRAALSRQKLDHVTDTHYVGLQFPDPAHPNTLHWVDEAGKVGEQLPLEDPDVYCPYSAIGNVTGELVYAHYGRPEDLQDLRARGVDPVGRLLLVRVGVISFAQKVTNAQDFGAQGVLIYPEPADFSQDPPKPSLSSQQAVYGHVHLGTGDPYTPGFPSFNQTQFPPVASSGLPSIPAQPISADIASRLLRKLKGPVAPQEWQGSLLGSPYHLGPGPRLRLVVNNHRTSTPINNIFGCIEGRSEPDHYVVIGAQRDAWGPGAAKSAVGTAILLELVRTFSSMVSNGFRPRRSLLFISWDGGDFGSVGSTEWLEGYLSVLHLKAVVYVSLDNAVLGDDKFHAKTSPLLTSLIESVLKQVDSPNHSGQTLYEQVVFTNPSWDAEVIRPLPMDSSAYSFTAFVGVPAVEFSFMEDDQAYPFLHTKEDTYENLHKVLQGRLPAVAQAVAQLAGQLLIRLSHDRLLPLDFGRYGDVVLRHIGNLNEFSGDLKARGLTLQWVYSARGDYIRAAEKLRQEIYSSEERDERLTRMYNVRIMRVEFYFLSQYVSPADSPFRHIFMGRGDHTLGALLDHLRLLRSNSSGTPGATSSTGFQESRFRRQLALLTWTLQGAANALSGDVWNIDNNF

SEQ ID NO: 4 - protein, 798 aa, Mus Musculus
MEQRWGLLRRVQQWSPRPSQTIYRRVEGPQLEHLEEEDREEGAELPAQFCPMELKGPEHLGSCPGRSIPIPWAAAGRKAAPYLVLITLLIFTGAFLLGYVAFRGSCQACGDSVLVVDEDVNPEDSGRTTLYWSDLQAMFLRFLGEGRMEDTIRLTSLRERVAGSARMATLVQDILDKLSRQKLDHVWTDTHYVGLQFPDPAHANTLHWVDADGSVQEQLPLEDPEVYCPYSATGNATGKLVYAHYGRSEDLQDLKAKGVELAGSLLLVRVGITSFAQKVAVAQDFGAQGVLIYPDPSDFSQDPHKPGLSSHQAVYGHVHLGTGDPYTPGFPSFNQTQFPPVESSGLPSIPAQPISADIADQLLRKLTGPVAPQEWKGHLSGSPYRLGPGPDLRLVVNNHRVSTPISNIFACIEGFAEPDHYVVIGAQRDAWGPGAAKSAVGTAILLELVRTFSSMVSNGFRPRRSLLFISWDGGDFGSVGATEWLEGYLSVLHLKAVVYVSLDNSVLGDGKFHAKTSPLLVSLIENILKQVDSPNHSGQTLYEQVALTHPSWDAEVIQPLPMDSSAYSFTAFAGVPAVEFSFMEDDRVYPFLHTKEDTYENLHKMLRGRLPAVVQAVAQLAGQLLIRLSHDHLLPLDFGRYGDVVLRHIGNLNEFSGDLKERGLTLQWVYSARGDYIRAAEKLRKEIYSSERNDERLMRMYNVRIMRVEFYFLSQYVSPADSPFRHIFLGQGDHTLGALVDHLRMLRADGSGAASSRLTAGLGFQESRFRRQLALLTWTLQGAANALSGDVWNIDNNF

SEQ ID NO: 5 - protein, 94 aa, Homo Sapien
YCPYSAIGNVTGELVYAHYGRPEDLQDLRARGVDPVGRLLLVRVGVISFAQKVTNAQDFGAQGVLIYPEPADFSQDPPKPSLSSQQAVYGHVHL

SEQ ID NO: 6 - protein, 186 aa, Homo Sapien
GRSEPDHYVVIGAQRDAWGPGAAKSAVGTAILLELVRTFSSMVSNGFRPRRSLLFISWDGGDFGSVGSTEWLEGYLSVLHLKAVVYVSLDNAVLGDDKFHAKTSPLLTSLIESVLKQVDSPNHSGQTLYEQVVFTNPSWDAEVIRPLPMDSSAYSFTAFVGVPAVEFSFMEDDQAYPFLHTKEDTY

SEQ ID NO: 7 - protein, 126 aa, Homo Sapien
LKARGLTLQWVYSARGDYIRAAEKLRQEIYSSEERDERLTRMYNVRIMRVEFYFLSQYVSPADSPFRHIFMGRGDHTLGALLDHLRLLRSNSSGTPGATSSTGFQESRFRRQLALLTWTLQGAANA

SEQ ID NO: 8 - protein, 2538 aa, Homo Sapien
GTTCGTTGCAACAAATTGATGAGCAATGCTTTTTTATAATGCCAACTTTGTACAAAAAAGTTGGCACCATGGAGCGGCTTTGGGGTCTATTCCAGAGAGCGCAACAACTGTCCCCAAGATCCTCTCAGACCGTCTACCAGCGTGTGGAAGGCCCCCGGAAAGGGCACCTGGAGGAGGAAGAGGAAGACGGGGAGGAGGGGGCGGAGACATTGGCCCACTTCTGCCCCATGGAGCTGAGGGGCCCTGAGCCCCTGGGCTCTAGACCCAGGCAGCCAAACCTCATTCCCTGGGCGGCAGCAGGACGGAGGGCTGCCCCCTACCTGGTCCTGACGGCCCTGCTGATCTTCACTGGGGCCTTCCTACTGGGCTACGTCGCCTTCCGAGGGTCCTGCCAGGCGTGCGGAGACTCTGTGTTGGTGGTCAGTGAGGATGTCAACTATGAGCCTGACCTGGATTTCCACCAGGGCAGACTCTACTGGAGCGACCTCCAGGCCATGTTCCTGCAGTTCCTGGGGGAGGGGCGCCTGGAGGACACCATCAGGCAAACCAGCCTTCGGGAACGGGTGGCAGGCTCGGCCGGGATGGCCGCTCTGACTCAGGACATTCGCGCGGCGCTCTCCCGCCAGAAGCTGGACCACGTGTGGACCGACACGCACTACGTGGGGCTGCAATTCCCGGATCCGGCTCACCCCAACACCCTGCACTGGGTCGATGAGGCCGGGAAGGTCGGAGAGCAGCTGCCGCTGGAGGACCCTGACGTCTACTGCCCCTACAGCGCCATCGGCAACGTCACGGGAGAGCTGGTGTACGCCCACTACGGGCGGCCCGAAGACCTGCAGGACCTGCGGGCCAGGGGCGTGGATCCAGTGGGCCGCCTGCTGCTGGTGCGCGTGGGGGTGATCAGCTTCGCCCAGAAGGTGACCAATGCTCAGGACTTCGGGGCTCAAGGAGTGCTCATATACCCAGAGCCAGCGGACTTCTCCCAGGACCCACCCAAGCCAAGCCTGTCCAGCCAGCAGGCAGTGTATGGACATGTGCACCTGGGAACTGGAGACCCCTACACACCTGGCTTCCCTTCCTTCAATCAAACCCAGTTCCCTCCAGTTGCATCATCAGGCCTTCCCAGCATCCCAGCCCAGCCCATCAGTGCAGACATTGCCTCCCGCCTGCTGAGGAAGCTCAAAGGCCCTGTGGCCCCCCAAGAATGGCAGGGGAGCCTCCTAGGCTCCCCTTATCACCTGGGCCCCGGGCCACGACTTCGGCTAGTGGTCAACAATCACAGGACCTCCACCCCCATCAACAACATCTTCGGCTGCATCGAAGGCCGCTCAGAGCCAGATCACTACGTTGTCATCGGGGCCCAGAGGGATGCATGGGGCCCAGGAGCAGCTAAATCCGCTGTGGGGACGGCTATACTCCTGGAGCTGGTGCGGACCTTTTCCTCCATGGTGAGCAACGGCTTCCGGCCCCGCAGAAGTCTCCTCTTCATCAGCTGGGACGGTGGTGACTTTGGAAGCGTGGGCTCCACGGAGTGGCTAGAGGGCTACCTCAGCGTGCTGCACCTCAAAGCCGTAGTGTACGTGAGCCTGGACAACGCAGTGCTGGGGGATGACAAGTTTCATGCCAAGACCAGCCCCCTTCTGACAAGTCTCATTGAGAGTGTCCTGAAGCAGGTGGATTCTCCCAACCACAGTGGGCAGACTCTCTATGAACAGGTGGTGTTCACCAATCCCAGCTGGGATGCTGAGGTGATCCGGCCCCTACCCATGGACAGCAGTGCCTATTCCTTCACGGCCTTTGTGGGAGTCCCTGCCGTCGAGTTCTCCTTTATGGAGGACGACCAGGCCTACCCATTCCTGCACACAAAGGAGGACACTTATGAGAACCTGCATAAGGTGCTGCAAGGCCGCCTGCCCGCCGTGGCCCAGGCCGTGGCCCAGCTCGCAGGGCAGCTCCTCATCCGGCTCAGCCACGATCGCCTGCTGCCCCTCGACTTCGGCCGCTACGGGGACGTCGTCCTCAGGCACATCGGGAACCTCAACGAGTTCTCTGGGGACCTCAAGGCCCGCGGGCTGACCCTGCAGTGGGTGTACTCGGCGCGGGGGGACTACATCCGGGCGGCGGAAAAGCTGCGGCCGGAGATCTACAGCTCGGAGGAGAGAGACGAGCGACTGACACGCATGTACAACGTGCGCATAATGCGGGTGGAGTTCTACTTCCTTTCCCAGTACGTGTCGCCAGCCGACTCCCCGTTCCGCCACATCTTCATGGGCCGTGGAGACCACACGCTGGGCGCCCTGCTGGACCACCTGCGGCTGCTGCGCTCCAACAGCTCCGGGACCCCCGGGGCCACCTCCTCCACTGGCTTCCAGGAGAGCCGTTTCCGGCGTCAGCTAGCCCTGCTCACCTGGACGCTGCAAGGGGCAGCCAATGCGCTTAGCGGGGATGTCTGGAACATTGATAACAACTTCTTGCCAACTTTCTTGTACAAAGTTGGCATTATAAGAAAGCATTGCTTATCAATTTGTTGCAACGAAC

SEQ ID NO: 9 - protein, 3596 aa, Mus Musculus
GAGTCTCCTGGGAGCATGGTCCAAGAAACCCAGAGACCTGTTGCTGAGCTGAACTTGGCTGCTGTGTCTTCCCACTCAGGACTCGGCTTTGACAGGCACGAGGCAGGGACTGGGGTACTGGTGAGCCCCTACCTCTCAGATCTTTCTGGACCTGGCTGCAGGTCCTGGTGTCTTCGTCGCGGCTTGGATTTCAAACTGGAGGAGTTCAGGAGGGGGCACAAGCATGGAGCAACGTTGGGGTCTACTTCGGAGAGTGCAACAGTGGTCCCCAAGACCCTCTCAGACCATCTACAGACGCGTGGAAGGCCCTCAGCTGGAGCACCTGGAGGAGGAAGACAGGGAGGAAGGGGCGGAGCTTCCTGCCCAGTTCTGCCCCATGGAACTCAAAGGCCCTGAGCACTTAGGCTCCTGTCCCGGGAGTCAATTCCCATACCCTGGGCTGCAGCAGGTCGAAAGGCTGCCCCCTATCTGGTCCTGATCACCCTGCTAATCTTCACTGGGGCCTTCCTCCTAGGCTACGTGGCCTTTCGAGGGTCCTGCCAGGCGTGTGGGGACTCCGTGTTGGTGGTCGATGAAGATGTCAACCCTGAGGACTCCGGCCGGACCACGTTGTACTGGAGCGACCTCCAGGCCATGTTTCTCCGGTTCCTTGGGGAGGGGCGCATGGAAGACACCATCAGGCTGACCAGCCTCCGGGAACGCGTGGCTGGCTCAGCCAGAATGGCCACCCTGGTCCAAGATATCCTCGATAAGCTCTCGCGCCAGAAGCTGGACCACGTGTGGACTGACACGCACTACGTGGGACTTCAGTTCCCAGATCCGGCTCACGCTAACACCCTGCACTGGGTGGATGCAGACGGGAGCGTCCAGGAGCAGCTACCGCTGGAGGATCCGGAAGTCTACTGTCCCTACAGCGCCACCGGCAACGCCACGGGCAAGCTGGTGTACGCCCACTACGGGCGGTCGGAGGACCTACAGGACCTAAAAGCCAAGGGCGTGGAGCTGGCCGGCAGCCTCCTGCTAGTGCGAGTTGGAATTACTAGCTTCGCCCAGAAGGTAGCCGTTGCCCAGGACTTTGGGGCTCAAGGAGTGCTGATATACCCTGACCCATCAGACTTCTCCCAGGATCCCCACAAGCCAGGCCTGTCTAGCCACCAGGCTGTGTACGGACATGTGCACCTGGGAACTGGAGACCCTTACACACCTGGCTTCCCGTCCTTCAATCAAACCCAGTTCCCTCCAGTAGAATCATCAGGCCTTCCCAGCATCCCCGCCCAGCCCATCAGTGCTGACATTGCTGATCAATTGCTCAGGAAACTCACAGGCCCCGTGGCTCCCCAGGAGTGGAAAGGTCACCTCTCAGGCTCTCCTTATCGGCTGGGACCTGGGCCCGACTTACGCCTTGTGGTCAACAACCACAGAGTCTCTACCCCCATCAGTAACATCTTTGCGTGCATCGAGGGCTTTGCAGAGCCAGATCACTATGTTGTCATTGGGGCCCAGAGGGATGCATGGGGCCCAGGAGCAGCCAAGTCTGCAGTGGGGACTGCCATCCTGCTGGAGCTGGTTCGGACCTTCTCTTCCATGGTCAGCAATGGGTTCAGACCTCGAAGAAGTCTTTTGTTCATCAGCTGGGACGGAGGTGACTTTGGCAGCGTGGGAGCCACAGAGTGGTTGGAGGGCTACCTCAGCGTGCTACACCTCAAAGCTGTTGTGTACGTGAGCCTGGACAACTCCGTGTTGGGAGATGGCAAATTCCATGCTAAGACCAGCCCCCTTCTCGTCAGCCTCATTGAGAATATCTTGAAGCAGGTGGACTCCCCTAACCATAGTGGACAGACCCTCTATGAACAAGTGGCACTCACCCACCCCAGCTGGGATGCTGAAGTGATTCAGCCCCTGCCCATGGACAGCAGTGCATATTCCTTCACAGCCTTTGCGGGGGTCCCAGCTGTGGAGTTCTCCTTCATGGAGGATGATCGGGTGTACCCATTCCTGCACACGAAGGAGGACACATATGAGAATCTGCACAAGATGCTGCGAGGTCGCCTGCCCGCCGTGGTCCAGGCAGTGGCTCAGCTCGCGGGCCAGCTCCTCATCCGACTGAGCCACGATCACCTACTGCCGCTAGACTTCGGCCGCTATGGAGACGTGGTTCTCAGGCACATCGGCAACCTCAATGAGTTCTCTGGGGACCTCAAGGAGCGCGGGCTGACCCTGCAGTGGGTGTACTCTGCAAGGGGGGACTACATCCGTGCGGCGGAAAAGCTGCGGAAGGAGATTTACAGCTCGGAGCGGAACGATGAGCGTCTGATGCGCATGTACAACGTGCGCATCATGAGGGTGGAGTTCTACTTCCTGTCCCAGTATGTGTCGCCAGCCGACTCCCCATTCCGCCACATTTTCCTAGGCCAAGGCGACCACACTTTGGGTGCCCTGGTAGACCACCTGCGGATGCTGCGCGCCGATGGCTCAGGAGCCGCCTCTTCCCGGTTGACAGCAGGTCTGGGCTTCCAGGAGAGTCGCTTCCGGCGCCAGCTGGCGCTGCTCACCTGGACACTGCAGGGGGCAGCCAACGCTCTCAGTGGCGACGTTTGGAACATTGACAATAACTTTTGAAGCCAAAAGCCCTCCATGGGCCCCACGTGATTCTCCTTTCTCCCTCTTTGAGTGGTGCAGGCAAAGGAGGTGCCTGAGATTGTAACCTATTCTTAACACCCTTGGTCCTGCAATGCTGGTGCGCCATATTTTCTCAGTGTGGTTGTCATGCCGTTGCTTACCCAGAAAGCGGTTTTCTTCCCATCACAGGCCCTTCTGTCTTCAGGAGCAAAGTTCCCCATATCTAGAGACTATCTAGATGCTGGGATCTGATCAGCTCTCTTAGAGAGTGAGATGGACAGCGTCATTATTTTATGACACATGAGCTACGGTATGTGAGCAGCCCAAGGGGATTAGATGTCAATAAACCAATTGTAACCCCTGTTGTCCATACGCAATTTAGCTTCCTCTTCATGCCGTACCCACTCCTCATATCCGCCTTGAGACTAGGGAAGAAGGCACAGAAGGCACCTGACAGCATGCTTGCAAGATGCTATCCACATGGGAAAAATAACTGTTCTGATGTCTAAGAAAACTGCCTAAAGATAATGGATAGGAGGTGGGGCAGTGGGGATAACTCATCAGGAATGGGTGATTGCGGCCAAGCCTGATGACCTGAGTTTAATCCCCAGGACCAACATGGCAAAAGGAGAGAACTAGTTCCCACAAGTTTTCCTATATCCTCCAAATGTATGCCCATAAAAGCACAAATAGATAAATGTTTTTGCTTTTGTTTTTTAAAGTGGCTTTGTGGTTAAGAGCACTGGATGCCATTCTAGAAGACACCGGTTCGATTCCCAGCACCCACATGGCCGCTTACAACTGTCTGTAACTCCAGTTGCTGGGGATCAGATGCCCTCTTCTGGTATGGTGTACGACTGCATGCATGTAGTATACATACAAGCAGGCAAAATACCCATACATGTAAAATTTTTAAAAAATAGTTTAAATTATAAATTAATTTAAAGAACAAATAAAAGATTAATGCCTTTAATCCC

SEQ ID NO: 10 - protein, 707 aa, Homo Sapien
AFRGSCQACGDSVLVVSEDVNYEPDLDFHQGRLYWSDLQAMFLQFLGEGRLEDTIRQTSLRERVAGSAGMAALTQDIRAALSRQKLDHVWTDTHYVGLQFPDPAHPNTLHWVDEAGKVGEQLPLEDPDVYCPYSAIGNVTGELVYAHYGRPEDLQDLRARGVDPVGRLLLVRVGVISFAQKVTNAQDFGAQGVLIYPEPADFSQDPPKPSLSSQQAVYGHVHLGTGDPYTPGFPSFNQTQFPPVASSGLPSIPAQPISADIASRLLRKLKGPVAPQEWQGSLLGSPYHLGPGPRLRLVVNNHRTSTPINNIFGCIEGRSEPDHYVVIGAQRDAWGPGAAKSAVGTAILLELVRTFSSMVSNGFRPRRSLLFISWDGGDFGSVGSTEWLEGYLSVLHLKAVVYVSLDNAVLGDDKFHAKTSPLLTSLIESVLKQVDSPNHSGQTLYEQVVFTNPSWDAEVIRPLPMDSSAYSFTAFVGVPAVEFSFMEDDQAYPFLHTKEDTYENLHKVLQGRLPAVAQAVAQLAGQLLIRLSHDRLLPLDFGRYGDVVLRHIGNLNEFSGDLKARGLTLQWVYSARGDYIRAAEKLRQEIYSSEERDERLTRMYNVRIMRVEFYFLSQYVSPADSPFRHIFMGRGDHTLGALLDHLRLLRSNSSGTPGATSSTGFQESRFRRQLALLTWTLQGAANALSGDVWNIDGGGGSHHHHHH

SEQ ID NO: 11 - protein, 933 aa, Homo Sapien
EPKSCDKTHTCPPCPAPELLGGPSVFLFPPKPKDTLMISRTPEVTCVVVDVSHEDPEVKFNWYVDGVEVHNAKTKPREEQYNSTYRVVSVLTVLHQDWLNGKEYKCKVSNKALPAPIEKTISKAKGQPREPQVYTLPPSRDELTKNQVSLTCLVKGFYPSDIAVEWESNGQPENNYKTTPPVLDSDGSFFLYSKLTVDKSRWQQGNVFSCSVMHEALHNHYTQKSLSLSPGKIEGRRGSCQACGDSVLVVSEDVNYEPDLDFHQGRLYWSDLQAMFLQFLGEGRLEDTIRQTSLRERVAGSAGMAALTQDIRAALSRQKLDHVWTDTHYVGLQFPDPAHPNTLHWVDEAGKVGEQLPLEDPDVYCPYSAIGNVTGELVYAHYGRPEDLQDLRARGVDPVGRLLLVRVGVISFAQKVTNAQDFGAQGVLIYPEPADFSQDPPKPSLSSQQAVYGHVHLGTGDPYTPGFPSFNQTQFPPVASSGLPSIPAQPISADIASRLLRKLKGPVAPQEWQGSLLGSPYHLGPGPRLRLVVNNHRTSTPINNIFGCIEGRSEPDHYVVIGAQRDAWGPGAAKSAVGTAILLELVRTFSSMVSNGFRPRRSLLFISWDGGDFGSVGSTEWLEGYLSVLHLKAVVYVSLDNAVLGDDKFHAKTSPLLTSLIESVLKQVDSPNHSGQTLYEQVVFTNPSWDAEVIRPLPMDSSAYSFTAFVGVPAVEFSFMEDDQAYPFLHTKEDTYENLHKVLQGRLPAVAQAVAQLAGQLLIRLSHDRLLPLDFGRYGDVVLRHIGNLNEFSGDLKARGLTLQWVYSARGDYIRAAEKLRQEIYSSEERDERLTRMYNVRIMRVEFYFLSQYVSPADSPFRHIFMGRGDHTLGALLDHLRLLRSNSSGTPGATSSTGFQESRFRRQLALLTWTLQGAANALSGDVWNIDNNF

SEQ ID NO: 12 - protein, 933 aa, Homo Sapien
RGSCQACGDSVLVVSEDVNYEPDLDFHQGRLYWSDLQAMFLQFLGEGRLEDTIRQTSLRERVAGSAGMAALTQDIRAALSRQKLDHVWTDTHYVGLQFPDPAHPNTLHWVDEAGKVGEQLPLEDPDVYCPYSAIGNVTGELVYAHYGRPEDLQDLRARGVDPVGRLLLVRVGVISFAQKVTNAQDFGAQGVLIYPEPADFSQDPPKPSLSSQQAVYGHVHLGTGDPYTPGFPSFNQTQFPPVASSGLPSIPAQPISADIASRLLRKLKGPVAPQEWQGSLLGSPYHLGPGPRLRLVVNNHRTSTPINNIFGCIEGRSEPDHYVVIGAQRDAWGPGAAKSAVGTAILLELVRTFSSMVSNGFRPRRSLLFISWDGGDFGSVGSTEWLEGYLSVLHLKAVVYVSLDNAVLGDDKFHAKTSPLLTSLIESVLKQVDSPNHSGQTLYEQVVFTNPSWDAEVIRPLPMDSSAYSFTAFVGVPAVEFSFMEDDQAYPFLHTKEDTYENLHKVLQGRLPAVAQAVAQLAGQLLIRLSHDRLLPLDFGRYGDVVLRHIGNLNEFSGDLKARGLTLQWVYSARGDYIRAAEKLRQEIYSSEERDERLTRMYNVRIMRVEFYFLSQYVSPADSPFRHIFMGRGDHTLGALLDHLRLLRSNSSGTPGATSSTGFQESRFRRQLALLTWTLQGAANALSGDVWNIDNNFIEGREPKSCDKTHTCPPCPAPELLGGPSVFLFPPKPKDTLMISRTPEVTCVVVDVSHEDPEVKFNWYVDGVEVHNAKTKPREEQYNSTYRVVSVLTVLHQDWLNGKEYKCKVSNKALPAPIEKTISKAKGQPREPQVYTLPPSRDELTKNQVSLTCLVKGFYPSDIAVEWESNGQPENNYKTTPPVLDSDGSFFLYSKLTVDKSRWQQGNVFSCSVMHEALHNHYTQKSLSLSPGK

SEQ ID NO: 13 - DNA, 19 bp, synthetic construct
  misc_feature 1..19: note = Primer
  source 1..19: mol_type = other DNA
atctggcaccacaccttct

SEQ ID NO: 14 - DNA, 20 bp, synthetic construct
  misc_feature 1..20: note = Primer
  source 1..20: mol_type = other DNA
ggggtgttgaaggtctcaaa

SEQ ID NO: 15 - DNA, 20 bp, synthetic construct
  misc_feature 1..20: note = Primer
  source 1..20: mol_type = other DNA
gcagtgatggaggaaaatgc

SEQ ID NO: 16 - DNA, 20 bp, synthetic construct
  misc_feature 1..20: note = Primer
  source 1..20: mol_type = other DNA
attcaaggtggggaggtagc

SEQ ID NO: 17 - DNA, 20 bp, synthetic construct
  misc_feature 1..20: note = Primer
  source 1..20: mol_type = other DNA
cgctccacaaacgagaaaag

SEQ ID NO: 18 - DNA, 20 bp, synthetic construct
  misc_feature 1..20: note = Primer
  source 1..20: mol_type = other DNA
cagtcattccaccccacatc

SEQ ID NO: 19 - DNA, 20 bp, synthetic construct
  misc_feature 1..20: note = Primer
  source 1..20: mol_type = other DNA
ctcaagggagtggagattgg

SEQ ID NO: 20 - DNA, 20 bp, synthetic construct
  misc_feature 1..20: note = Primer
  source 1..20: mol_type = other DNA
cttctgcgggtcaaggtatg

SEQ ID NO: 21 - DNA, 20 bp, synthetic construct
  misc_feature 1..20: note = Primer
  source 1..20: mol_type = other DNA
tagcaatctgtgggtggtga

SEQ ID NO: 22 - DNA, 20 bp, synthetic construct
  misc_feature 1..20: note = Primer
  source 1..20: mol_type = other DNA
gaagggctgcttgtcgtaag

SEQ ID NO: 23 - DNA, 21 bp, synthetic construct
  misc_feature 1..21: note = Primer
  source 1..21: mol_type = other DNA
tccttcgatggaccggttacc

SEQ ID NO: 24 - DNA, 20 bp, synthetic construct
  misc_feature 1..20: note = Primer
  source 1..20: mol_type = other DNA
gtggagccgctgctgacatc

SEQ ID NO: 25 - DNA, 20 bp, synthetic construct
  misc_feature 1..20: note = Primer
  source 1..20: mol_type = other DNA
gaggggaaattgaggaaagc

SEQ ID NO: 26 - DNA, 20 bp, synthetic construct
  misc_feature 1..20: note = Primer
  source 1..20: mol_type = other DNA
agccttcttgtcctttggtg

SEQ ID NO: 27 - DNA, 24 bp, synthetic construct
  misc_feature 1..24: note = Primer
  source 1..24: mol_type = other DNA
tgtcattctccttgtgttcctttg

SEQ ID NO: 28 - DNA, 28 bp, synthetic construct
  misc_feature 1..28: note = Primer
  source 1..28: mol_type = other DNA
agagctttcagattcagtattgtcgtat

SEQ ID NO: 29 - DNA, 20 bp, synthetic construct
  misc_feature 1..20: note = Primer
  source 1..20: mol_type = other DNA
cccactggaccgatccgcca

SEQ ID NO: 30 - DNA, 20 bp, synthetic construct
  misc_feature 1..20: note = Primer
  source 1..20: mol_type = other DNA
tgctctcggttccccagggg

SEQ ID NO: 31 - DNA, 20 bp, synthetic construct
  misc_feature 1..20: note = Primer
  source 1..20: mol_type = other DNA
tctgggggatgctgggcacc

SEQ ID NO: 32 - DNA, 20 bp, synthetic construct
  misc_feature 1..20: note = Primer
  source 1..20: mol_type = other DNA
gcttgggcatctcccggagc

SEQ ID NO: 33 - DNA, 20 bp, synthetic construct
  misc_feature 1..20: note = Primer
  source 1..20: mol_type = other DNA
caaataaagtgcccgtggtg

SEQ ID NO: 34 - DNA, 20 bp, synthetic construct
  misc_feature 1..20: note = Primer
  source 1..20: mol_type = other DNA
tcgtcgctgtaggtgatgag

SEQ ID NO: 35 - DNA, 24 bp, synthetic construct
  misc_feature 1..24: note = Primer
  source 1..24: mol_type = other DNA
ggaagaaaaccattgccaattatt

SEQ ID NO: 36 - DNA, 18 bp, synthetic construct
  misc_feature 1..18: note = Primer
  source 1..18: mol_type = other DNA
cgcctgctgaggtttgga

SEQ ID NO: 37 - DNA, 24 bp, synthetic construct
  misc_feature 1..24: note = Primer
  source 1..24: mol_type = other DNA
aagtcagggtgattgggggaatcc

SEQ ID NO: 38 - DNA, 24 bp, synthetic construct
  misc_feature 1..24: note = Primer
  source 1..24: mol_type = other DNA
aaaccatctcctcggatagggcac

SEQ ID NO: 39 - DNA, 20 bp, synthetic construct
  misc_feature 1..20: note = Primer
  source 1..20: mol_type = other DNA
attctcggctgtctcctcct

SEQ ID NO: 40 - DNA, 20 bp, synthetic construct
  misc_feature 1..20: note = Primer
  source 1..20: mol_type = other DNA
ccctgaggtaggtcgtagaa

SEQ ID NO: 41 - DNA, 20 bp, synthetic construct
  misc_feature 1..20: note = Primer
  source 1..20: mol_type = other DNA
cgtgcctcatctgcctactt

SEQ ID NO: 42 - DNA, 20 bp, synthetic construct
  misc_feature 1..20: note = Primer
  source 1..20: mol_type = other DNA
tgacctctgtggcatcattc

SEQ ID NO: 43 - DNA, 20 bp, synthetic construct
  misc_feature 1..20: note = Primer
  source 1..20: mol_type = other DNA
ggacatcagccagaagcaag

SEQ ID NO: 44 - DNA, 20 bp, synthetic construct
  misc_feature 1..20: note = Primer
  source 1..20: mol_type = other DNA
ggacagggggtagagaggag

SEQ ID NO: 45 - DNA, 21 bp, synthetic construct
  misc_feature 1..21: note = Primer
  source 1..21: mol_type = other DNA
gccatgtttctcccggttcct

SEQ ID NO: 46 - DNA, 18 bp, synthetic construct
  misc_feature 1..18: note = Primer
  source 1..18: mol_type = other DNA
tggcgcgagagcttatcg

SEQ ID NO: 47 - DNA, 21 bp, synthetic construct
  misc_feature 1..21: note = Primer
  source 1..21: mol_type = other DNA
cctggcccctagtgtgatttc

SEQ ID NO: 48 - DNA, 18 bp, synthetic construct
  misc_feature 1..18: note = Primer
  source 1..18: mol_type = other DNA
tggcgcgagagcttatcg

SEQ ID NO: 49 - DNA, 19 bp, synthetic construct
  misc_feature 1..19: note = Primer
  source 1..19: mol_type = other DNA
gacctccatagaagacacc

SEQ ID NO: 50 - DNA, 21 bp, synthetic construct
  misc_feature 1..21: note = Primer
  source 1..21: mol_type = other DNA
aacccgttgatgtccacttgc

SEQ ID NO: 51 - protein, 990 aa, Homo Sapien
GCCTCCACCAAGGGCCCATCGGTCTTCCCCCTGGCACCCTCCTCCAAGAGCACCTCTGGGGGCACAGCGGCCCTGGGCTGCCTGGTCAAGGACTACTTCCCCGAACCGGTGACGGTGTCGTGGAACTCAGGCGCCCTGACCAGCGGCGTGCACACCTTCCCGGCTGTCCTACAGTCCTCAGGACTCTACTCCCTCAGCAGCGTGGTGACCGTGCCCTCCAGCAGCTTGGGCACCCAGACCTACATCTGCAACGTGAATCACAAGCCCAGCAACACCAAGGTGGACAAGAAAGTTGAGCCCAAATCTTGTGACAAAACTCACACATGCCCACCGTGCCCAGCACCTGAACTCCTGGGGGGACCGTCAGTCTTCCTCTTCCCCCCAAAACCCAAGGACACCCTCATGATCTCCCGGACCCCTGAGGTCACATGCGTGGTGGTGGACGTGAGCCACGAAGACCCTGAGGTCAAGTTCAACTGGTACGTGGACGGCGTGGAGGTGCATAATGCCAAGACAAAGCCGCGGGAGGAGCAGTACAACAGCACGTACCGGGTGGTCAGCGTCCTCACCGTCCTGCACCAGGACTGGCTGAATGGCAAGGAGTACAAGTGCAAGGTCTCCAACAAAGCCCTCCCAGCCCCCATCGAGAAAACCATCTCCAAAGCCAAAGGGCAGCCCCGAGAACCACAGGTGTACACCCTGCCCCCATCCCGGGATGAGCTGACCAAGAACCAGGTCAGCCTGACCTGCCTGGTCAAAGGCTTCTATCCCAGCGACATCGCCGTGGAGTGGGAGAGCAATGGGCAGCCGGAGAACAACTACAAGACCACGCCTCCCGTGCTGGACTCCGACGGCTCCTTCTTCCTCTACAGCAAGCTCACCGTGGACAAGAGCAGGTGGCAGCAGGGGAACGTCTTCTCATGCTCCGTGATGCATGAGGCTCTGCACAACCACTACACGCAGAAGAGCCTCTCCCTGTCTCCGGGTAAA

SEQ ID NO: 52 - protein, 330 aa, Homo Sapien [sequence omitted]

SEQ ID NO: 53 - protein, 990 aa, Homo Sapien
GCCTCCACCAAGGGCCCATCGGTCTTCCCCCTGGCACCCTCCTCCAAGAGCACCTCTGGGGGCACAGCGGCCCTGGGCTGCCTGGTCAAGGACTACTTCCCCGAACCGGTGACGGTGTCGTGGAACTCAGGCGCCCTGACCAGCGGCGTGCACACCTTCCCGGCTGTCCTACAGTCCTCAGGACTCTACTCCCTCAGCAGCGTGGTGACCGTGCCCTCCAGCAGCTTGGGCACCCAGACCTACATCTGCAACGTGAATCACAAGCCCAGCAACACCAAGGTGGACAAGAAAGTTGAGCCCAAATCTTGTGACAAAACTCACACATGCCCACCGTGCCCAGCACCTGAACTCCTGGGGGGACCGTCAGTCTTCCTCTTCCCCCCAAAACCCAAGGACACCCTCATGATCTCCCGGACCCCTGAGGTCACATGCGTGGTGGTGGACGTGAGCCACGAAGACCCTGAGGTCAAGTTCAACTGGTACGTGGACGGCGTGGAGGTGCATAATGCCAAGACAAAGCCGCGGGAGGAGCAGTACAACAGCACGTACCGTGTGGTCAGCGTCCTCACCGTCCTGCACCAGGACTGGCTGAATGGCAAGGAGTACAAGTGCAAGGTCTCCAACAAAGCCCTCCCAGCCCCCATCGAGAAAACCATCTCCAAAGCCAAAGGGCAGCCCCGAGAACCACAGGTGTACACCCTGCCCCCATCCCGGGATGAGCTGACCAAGAACCAGGTCAGCCTGACCTGCCTGGTCAAAGGCTTCTATCCCAGCGACATCGCCGTGGAGTGGGAGAGCAATGGGCAGCCGGAGAACAACTACAAGACCACGCCTCCCGTGCTGGACTCCGACGGCTCCTTCTTCCTCTACAGCAAGCTCACCGTGGACAAGAGCAGGTGGCAGCAGGGGAACGTCTTCTCATGCTCCGTGATGCATGAGGCTCTGCACAACCACTACACGCAGAAGAGCCTCTCCCTGTCTCCGGGTAAA

SEQ ID NO: 54 - protein, 330 aa, Homo Sapien [sequence omitted]

SEQ ID NO: 55 - protein, 990 aa, Homo Sapien
GCCTCCACCAAGGGCCCATCGGTCTTCCCCCTGGCACCCTCCTCCAAGAGCACCTCTGGGGGCACAGCGGCCCTGGGCTGCCTGGTCAAGGACTACTTCCCCGAACCGGTGACGGTGTCGTGGAACTCAGGCGCCCTGACCAGCGGCGTGCACACCTTCCCGGCTGTCCTACAGTCCTCAGGACTCTACTCCCTCAGCAGCGTGGTGACCGTGCCCTCCAGCAGCTTGGGCACCCAGACCTACATCTGCAACGTGAATCACAAGCCCAGCAACACCAAGGTGGACAAGAGAGTTGAGCCCAAATCTTGTGACAAAACTCACACATGCCCACCGTGCCCAGCACCTGAACTCCTGGGGGGACCGTCAGTCTTCCTCTTCCCCCCAAAACCCAAGGACACCCTCATGATCTCCCGGACCCCTGAGGTCACATGCGTGGTGGTGGACGTGAGCCACGAAGACCCTGAGGTCAAGTTCAACTGGTACGTGGACGGCGTGGAGGTGCATAATGCCAAGACAAAGCCGCGGGAGGAGCAGTACAACAGCACGTACCGTGTGGTCAGCGTCCTCACCGTCCTGCACCAGGACTGGCTGAATGGCAAGGAGTACAAGTGCAAGGTCTCCAACAAAGCCCTCCCAGCCCCCATCGAGAAAACCATCTCCAAAGCCAAAGGGCAGCCCCGAGAACCACAGGTGTACACCCTGCCCCCATCCCGGGAGGAGATGACCAAGAACCAGGTCAGCCTGACCTGCCTGGTCAAAGGCTTCTATCCCAGCGACATCGCCGTGGAGTGGGAGAGCAATGGGCAGCCGGAGAACAACTACAAGACCACGCCTCCCGTGCTGGACTCCGACGGCTCCTTCTTCCTCTATAGCAAGCTCACCGTGGACAAGAGCAGGTGGCAGCAGGGGAACGTCTTCTCATGCTCCGTGATGCATGAGGCTCTGCACAACCACTACACGCAGAAGAGCCTCTCCCTGTCCCCGGGTAAA

SEQ ID NO: 56 - protein, 330 aa, Homo Sapien
ASTKGPSVFPLAPSSKSTSGGTAALGCLVKDYFPEPVTVSWNSGALTSGVHTFPAVLQSSGLYSLSSVVTVPSSSLGTQTYICNVNHKPSNTKVDKRVEPKSCDKTHTCPPCPAPELLGGPSVFLFPPKPKDTLMISRTPEVTCVVVDVSHEDPEVKFNWYVDGVEVHNAKTKPREEQYNSTYRVVSVLTVLHQDWLNGKEYKCKVSNKALPAPIEKTISKAKGQPREPQVYTLPPSREEMTKNQVSLTCLVKGFYPSDIAVEWESNGQPENNYKTTPPVLDSDGSFFLYSKLTVDKSRWQQGNVFSCSVMHEALHNHYTQKSLSLSPGK

SEQ ID NO: 57 - protein, 990 aa, Homo Sapien
GCCTCCACCAAGGGCCCATCGGTCTTCCCCCTGGCACCCTCCTCCAAGAGCACCTCTGGGGGCACAGCGGCCCTGGGCTGCCTGGTCAAGGACTACTTCCCCGAACCGGTGACGGTGTCGTGGAACTCAGGCGCCCTGACCAGCGGCGTGCACACCTTCCCGGCTGTCCTACAGTCCTCAGGACTCTACTCCCTCAGCAGCGTGGTGACCGTGCCCTCCAGCAGCTTGGGCACCCAGACCTACATCTGCAACGTGAATCACAAGCCCAGCAACACCAAGGTGGACAAGAAAGTTGAGCCCAAATCTTGTGACAAAACTCACACATGCCCACCGTGCCCAGCACCTGAACTCCTGGGGGGACCGTCAGTCTTCCTCTTCCCCCCAAAACCCAAGGACACCCTCATGATCTCCCGGACCCCTGAGGTCACATGCGTGGTGGTGGACGTGAGCCACGAAGACCCTGAGGTCAAGTTCAACTGGTACGTGGACGGCGTGGAGGTGCATAATGCCAAGACAAAGCCGCGGGAGGAGCAGTACAACAGCACGTACCGTGTGGTCAGCGTCCTCACCGTCCTGCACCAGGACTGGCTGAATGGCAAGGAGTACAAGTGCAAGGTCTCCAACAAAGCCCTCCCAGCCCCCATCGAGAAAACCATCTCCAAAGCCAAAGGGCAGCCCCGAGAACCACAGGTGTACACCCTGCCCCCATCCCGGGATGAGCTGACCAAGAACCAGGTCAGCCTGACCTGCCTGGTCAAAGGCTTCTATCCCAGCGACATCGCCGTGGAGTGGGAGAGCAATGGGCAGCCGGAGAACAACTACAAGACCACGCCTCCCGTGCTGGACTCCGACGGCTCCTTCTTCCTCTACAGCAAGCTCACCGTGGACAAGAGCAGGTGGCAGCAGGGGAACATCTTCTCATGCTCCGTGATGCATGAGGCTCTGCACAACCACTACACGCAGAAGAGCCTCTCCCTGTCTCCGGGTAAA

SEQ ID NO: 58 - protein, 330 aa, Homo Sapien
ASTKGPSVFPLAPSSKSTSGGTAALGCLVKDYFPEPVTVSWNSGALTSGVHTFPAVLQSSGLYSLSSVVTVPSSSLGTQTYICNVNHKPSNTKVDKKVEPKSCDKTHTCPPCPAPELLGGPSVFLFPPKPKDTLMISRTPEVTCVVVDVSHEDPEVKFNWYVDGVEVHNAKTKPREEQYNSTYRVVSVLTVLHQDWLNGKEYKCKVSNKALPAPIEKTISKAKGQPREPQVYTLPPSRDELTKNQVSLTCLVKGFYPSDIAVEWESNGQPENNYKTTPPVLDSDGSFFLYSKLTVDKSRWQQGNIFSCSVMHEALHNHYTQKSLSLSPGK

SEQ ID NO: 59 - protein, 990 aa, synthetic construct
  REGION 1..990: note = Synthetic Constant Region
GCCTCCACCAAGGGCCCATCGGTCTTCCCCCTGGCACCCTCCTCCAAGAGCACCTCTGGGGGCACAGCGGCCCTGGGCTGCCTGGTCAAGGACTACTTCCCCGAACCGGTGACGGTGTCGTGGAACTCAGGCGCCCTGACCAGCGGCGTGCACACCTTCCCGGCTGTCCTACAGTCCTCAGGACTCTACTCCCTCAGCAGCGTGGTGACCGTGCCCTCCAGCAGCTTGGGCACCCAGACCTACATCTGCAACGTGAATCACAAGCCCAGCAACACCAAGGTGGACAAGAAAGTGGAGCCCAAATCTTGTGACAAAACTCACACATGCCCACCGTGCCCAGCACCTGAACTCGCGGGGGCACCGTCAGTCTTCCTCTTCCCCCCAAAACCCAAGGACACCCTCATGATCTCCCGGACCCCTGAGGTCACATGCGTGGTGGTGGACGTGAGCCACGAAGACCCTGAGGTCAAGTTCAACTGGTACGTGGACGGCGTGGAGGTGCATAATGCCAAGACAAAGCCGCGGGAGGAGCAGTACAACAGCACGTACCGTGTGGTCAGCGTCCTCACCGTCCTGCACCAGGACTGGCTGAATGGCAAGGAGTACAAGTGCAAGGTCTCCAACAAAGCCCTCCCAGCCCCCATCGAGAAAACCATCTCCAAAGCCAAAGGGCAGCCCCGAGAACCACAGGTGTACACCCTGCCCCCATCCCGGGATGAGCTGACCAAGAACCAGGTCAGCCTGACCTGCCTGGTCAAAGGCTTCTATCCCAGCGACATCGCCGTGGAGTGGGAGAGCAATGGGCAGCCGGAGAACAACTACAAGACCACGCCTCCCGTGCTGGACTCCGACGGCTCCTTCTTCCTCTACAGCAAGCTCACCGTGGACAAGAGCAGGTGGCAGCAGGGGAACGTCTTCTCATGCTCCGTGATGCATGAGGCTCTGCACAACCACTACACGCAGAAGAGCCTCTCCCTGTCTCCGGGTAAA

SEQ ID NO: 60 - protein, 330 aa, Homo Sapien
ASTKGPSVFPLAPSSKSTSGGTAALGCLVKDYFPEPVTVSWNSGALTSGVHTFPAVLQSSGLYSLSSVVTVPSSSLGTQTYICNVNHKPSNTKVDKKVEPKSCDKTHTCPPCPAPELAGAPSVFLFPPKPKDTLMISRTPEVTCVVVDVSHEDPEVKFNWYVDGVEVHNAKTKPREEQYNSTYRVVSVLTVLHQDWLNGKEYKCKVSNKALPAPIEKTISKAKGQPREPQVYTLPPSRDELTKNQVSLTCLVKGFYPSDIAVEWESNGQPENNYKTTPPVLDSDGSFFLYSKLTVDKSRWQQGNVFSCSVMHEALHNHYTQKSLSLSPGK

SEQ ID NO: 61 - protein, 978 aa, Homo Sapien
GCCTCCACCAAGGGCCCATCGGTCTTCCCCCTGGCGCCCTGCTCCAGGAGCACCTCCGAGAGCACAGCCGCCCTGGGCTGCCTGGTCAAGGACTACTTCCCCGAACCGGTGACGGTGTCGTGGAACTCAGGCGCTCTGACCAGCGGCGTGCACACCTTCCCAGCTGTCCTACAGTCCTCAGGACTCTACTCCCTCAGCAGCGTGGTGACCGTGCCCTCCAGCAACTTCGGCACCCAGACCTACACCTGCAACGTAGATCACAAGCCCAGCAACACCAAGGTGGACAAGACAGTTGAGCGCAAATGTTGTGTCGAGTGCCCACCGTGCCCAGCACCACCTGTGGCAGGACCGTCAGTCTTCCTCTTCCCCCCAAAACCCAAGGACACCCTCATGATCTCCCGGACCCCTGAGGTCACGTGCGTGGTGGTGGACGTGAGCCACGAAGACCCCGAGGTCCAGTTCAACTGGTACGTGGACGGCGTGGAGGTGCATAATGCCAAGACAAAGCCACGGGAGGAGCAGTTCAACAGCACGTTCCGTGTGGTCAGCGTCCTCACCGTTGTGCACCAGGACTGGCTGAACGGCAAGGAGTACAAGTGCAAGGTCTCCAACAAAGGCCTCCCAGCCCCCATCGAGAAAACCATCTCCAAAACCAAAGGGCAGCCCCGAGAACCACAGGTGTACACCCTGCCCCCATCCCGGGAGGAGATGACCAAGAACCAGGTCAGCCTGACCTGCCTGGTCAAAGGCTTCTACCCCAGCGACATCGCCGTGGAGTGGGAGAGCAATGGGCAGCCGGAGAACAACTACAAGACCACACCTCCCATGCTGGACTCCGACGGCTCCTTCTTCCTCTACAGCAAGCTCACCGTGGACAAGAGCAGGTGGCAGCAGGGGAACGTCTTCTCATGCTCCGTGATGCATGAGGCTCTGCACAACCACTACACGCAGAAGAGCCTCTCCCTGTCTCCGGGTAAA

SEQ ID NO: 62 - protein, 326 aa, Homo Sapien
ASTKGPSVFPLAPCSRSTSESTAALGCLVKDYFPEPVTVSWNSGALTSGVHTFPAVLQSSGLYSLSSVVTVPSSNFGTQTYTCNVDHKPSNTKVDKTVERKCCVECPPCPAPPVAGPSVFLFPPKPKDTLMISRTPEVTCVVVDVSHEDPEVQFNWYVDGVEVHNAKTKPREEQFNSTFRVVSVLTVVHQDWLNGKEYKCKVSNKGLPAPIEKTISKTKGQPREPQVYTLPPSREEMTKNQVSLTCLVKGFYPSDIAVEWESNGQPENNYKTTPPMLDSDGSFFLYSKLTVDKSRWQQGNVFSCSVMHEALHNHYTQKSLSLSPGK

SEQ ID NO: 63 - protein, 978 aa, Homo Sapien
GCCTCCACCAAGGGCCCATCGGTCTTCCCCCTGGCGCCCTGCTCCAGGAGCACCTCCGAGAGCACAGCGGCCCTGGGCTGCCTGGTCAAGGACTACTTCCCCGAACCGGTGACGGTGTCGTGGAACTCAGGCGCTCTGACCAGCGGCGTGCACACCTTCCCGGCTGTCCTACAGTCCTCAGGACTCTACTCCCTCAGCAGCGTGGTGACCGTGACCTCCAGCAACTTCGGCACCCAGACCTACACCTGCAACGTAGATCACAAGCCCAGCAACACCAAGGTGGACAAGACAGTTGAGCGCAAATGTTGTGTCGAGTGCCCACCGTGCCCAGCACCACCTGTGGCAGGACCGTCAGTCTTCCTCTTCCCCCCAAAACCCAAGGACACCCTCATGATCTCCCGGACCCCTGAGGTCACGTGCGTGGTGGTGGACGTGAGCCACGAAGACCCCGAGGTCCAGTTCAACTGGTACGTGGACGGCATGGAGGTGCATAATGCCAAGACAAAGCCACGGGAGGAGCAGTTCAACAGCACGTTCCGTGTGGTCAGCGTCCTCACCGTCGTGCACCAGGACTGGCTGAACGGCAAGGAGTACAAGTGCAAGGTCTCCAACAAAGGCCTCCCAGCCCCCATCGAGAAAACCATCTCCAAAACCAAAGGGCAGCCCCGAGAACCACAGGTGTACACCCTGCCCCCATCCCGGGAGGAGATGACCAAGAACCAGGTCAGCCTGACCTGCCTGGTCAAAGGCTTCTACCCCAGCGACATCGCCGTGGAGTGGGAGAGCAATGGGCAGCCGGAGAACAACTACAAGACCACACCTCCCATGCTGGACTCCGACGGCTCCTTCTTCCTCTACAGCAAGCTCACCGTGGACAAGAGCAGGTGGCAGCAGGGGAACGTCTTCTCATGCTCCGTGATGCATGAGGCTCTGCACAACCACTACACACAGAAGAGCCTCTCCCTGTCTCCGGGTAAA

SEQ ID NO: 64 - protein, 326 aa, Homo Sapien
ASTKGPSVFPLAPCSRSTSESTAALGCLVKDYFPEPVTVSWNSGALTSGVHTFPAVLQSSGLYSLSSVVTVTSSNFGTQTYTCNVDHKPSNTKVDKTVERKCCVECPPCPAPPVAGPSVFLFPPKPKDTLMISRTPEVTCVVVDVSHEDPEVQFNWYVDGMEVHNAKTKPREEQFNSTFRVVSVLTVVHQDWLNGKEYKCKVSNKGLPAPIEKTISKTKGQPREPQVYTLPPSREEMTKNQVSLTCLVKGFYPSDIAVEWESNGQPENNYKTTPPMLDSDGSFFLYSKLTVDKSRWQQGNVFSCSVMHEALHNHYTQKSLSLSPGK

SEQ ID NO: 65 - protein, 978 aa, Homo Sapien
GCCTCCACCAAGGGCCCATCGGTCTTCCCCCTGGCGCCCTGCTCCAGGAGCACCTCCGAGAGCACAGCGGCCCTGGGCTGCCTGGTCAAGGACTACTTCCCCGAACCGGTGACGGTGTCGTGGAACTCAGGCGCTCTGACCAGCGGCGTGCACACCTTCCCAGCTGTCCTACAGTCCTCAGGACTCTACTCCCTCAGCAGCGTGGTGACCGTGCCCTCCAGCAGCTTGGGCACCCAGACCTACACCTGCAACGTAGATCACAAGCCCAGCAACACCAAGGTGGACAAGACAGTTGAGCGCAAATGTTGTGTCGAGTGCCCACCGTGCCCAGCACCACCTGTGGCAGGACCGTCAGTCTTCCTCTTCCCCCCAAAACCCAAGGACACCCTCATGATCTCCCGGACCCCTGAGGTCACGTGCGTGGTGGTGGACGTGAGCCACGAAGACCCCGAGGTCCAGTTCAACTGGTACGTGGACGGCGTGGAGGTGCATAATGCCAAGACAAAGCCACGGGAGGAGCAGTTCAACAGCACGTTCCGTGTGGTCAGCGTCCTCACCGTTGTGCACCAGGACTGGCTGAACGGCAAGGAGTACAAGTGCAAGGTCTCCAACAAAGGCCTCCCAGCCCCCATCGAGAAAACCATCTCCAAAACCAAAGGGCAGCCCCGAGAACCACAGGTGTACACCCTGCCCCCATCCCGGGAGGAGATGACCAAGAACCAGGTCAGCCTGACCTGCCTGGTCAAAGGCTTCTACCCCAGCGACATCGCCGTGGAGTGGGAGAGCAATGGGCAGCCGGAGAACAACTACAAGACCACACCTCCCATGCTGGACTCCGACGGCTCCTTCTTCCTCTACAGCAAGCTCACCGTGGACAAGAGCAGGTGGCAGCAGGGGAACGTCTTCTCATGCTCCGTGATGCATGAGGCTCTGCACAACCACTACACGCAGAAGAGCCTCTCCCTGTCTCCGGGTAAA

SEQ ID NO: 66 - protein, 326 aa, Homo Sapien
ASTKGPSVFPLAPCSRSTSESTAALGCLVKDYFPEPVTVSWNSGALTSGVHTFPAVLQSSGLYSLSSVVTVPSSSLGTQTYTCNVDHKPSNTKVDKTVERKCCVECPPCPAPPVAGPSVFLFPPKPKDTLMISRTPEVTCVVVDVSHEDPEVQFNWYVDGVEVHNAKTKPREEQFNSTFRVVSVLTVVHQDWLNGKEYKCKVSNKGLPAPIEKTISKTKGQPREPQVYTLPPSREEMTKNQVSLTCLVKGFYPSDIAVEWESNGQPENNYKTTPPMLDSDGSFFLYSKLTVDKSRWQQGNVFSCSVMHEALHNHYTQKSLSLSPGK

SEQ ID NO: 67 - protein, 922 aa, Homo Sapien
GCCTCCACCAAGGGCCCATCGGTCTTCCCCCTGGCGCCCTGCTCCAGGAGCACCTCCGAGAGCACAGCGGCCCTGGGCTGCCTGGTCAAGGACTACTTCCCCGAACCGGTGACGGTGTCGTGGAACTCAGGCGCTCTGACCAGCGGCGTGCACACCTTCCCGGCTGTCCTACAGTCCTCAGGACTCTACTCCCTCAGCAGCGTGGTGACCGTGCCCTCCAGCAACTTCGGCACCCAGACCTACACCTGCAACGTAGATCACAAGCCCAGCAACACCAAGGTGGGTGGCAGGACCGTCAGTCTTCCTCTTCCCCCCAAAACCCAAGGACACCCTCATGATCTCCCGGACCCCTGAGGTCACGTGCGTGGTGGTGGACGTGAGCCACGAAGACCCCGAGGTCCAGTTCAACTGGTACGTGGACGGCGTGGAGGTGCATAATGCCAAGACAAAGCCACGGGAGGAGCAGTTCAACAGCACGTTCCGTGTGGTCAGCGTCCTCACCGTCGTGCACCAGGACTGGCTGAACGGCAAGGAGTACAAGTGCAAGGTCTCCAACAAAGGCCTCCCAGCCCCCATCGAGAAAACCATCTCCAAAACCAAAGGGCAGCCCCGAGAACCACAGGTGTACACCCTGCCCCCATCCCGGGAGGAGATGACCAAGAACCAGGTCAGCCTGACCTGCCTGGTCAAAGGCTTCTACCCCAGCGACATCTCCGTGGAGTGGGAGAGCAATGGGCAGCCGGAGAACAACTACAAGACCACACCTCCCATGCTGGACTCCGACGGCTCCTTCTTCCTCTACAGCAAGCTCACCGTGGACAAGAGCAGGTGGCAGCAGGGGAACGTCTTCTCATGCTCCGTGATGCATGAGGCTCTGCACAACCACTACACACAGAAGAGCCTCTCCCTGTCTCCGGGTAAA

SEQ ID NO: 68 - protein, 326 aa, Homo Sapien
ASTKGPSVFPLAPCSRSTSESTAALGCLVKDYFPEPVTVSWNSGALTSGVHTFPAVLQSSGLYSLSSVVTVPSSNFGTQTYTCNVDHKPSNTKVDKTVERKCCVECPPCPAPPVAGPSVFLFPPKPKDTLMISRTPEVTCVVVDVSHEDPEVQFNWYVDGVEVHNAKTKPREEQFNSTFRVVSVLTVVHQDWLNGKEYKCKVSNKGLPAPIEKTISKTKGQPREPQVYTLPPSREEMTKNQVSLTCLVKGFYPSDISVEWESNGQPENNYKTTPPMLDSDGSFFLYSKLTVDKSRWQQGNVFSCSVMHEALHNHYTQKSLSLSPGK

SEQ ID NO: 69 - protein, 981 aa, Homo Sapien
GCTTCCACCAAGGGCCCATCCGTCTTCCCCCTGGCGCCCTGCTCCAGGAGCACCTCCGAGAGCACAGCCGCCCTGGGCTGCCTGGTCAAGGACTACTTCCCCGAACCGGTGACGGTGTCGTGGAACTCAGGCGCCCTGACCAGCGGCGTGCACACCTTCCCGGCTGTCCTACAGTCCTCAGGACTCTACTCCCTCAGCAGCGTGGTGACCGTGCCCTCCAGCAGCTTGGGCACGAAGACCTACACCTGCAACGTAGATCACAAGCCCAGCAACACCAAGGTGGACAAGAGAGTTGAGTCCAAATATGGTCCCCCATGCCCATCATGCCCAGCACCTGAGTTCCTGGGGGGACCATCAGTCTTCCTGTTCCCCCCAAAACCCAAGGACACTCTCATGATCTCCCGGACCCCTGAGGTCACGTGCGTGGTGGTGGACGTGAGCCAGGAAGACCCCGAGGTCCAGTTCAACTGGTACGTGGATGGCGTGGAGGTGCATAATGCCAAGACAAAGCCGCGGGAGGAGCAGTTCAACAGCACGTACCGTGTGGTCAGCGTCCTCACCGTCCTGCACCAGGACTGGCTGAACGGCAAGGAGTACAAGTGCAAGGTCTCCAACAAAGGCCTCCCGTCCTCCATCGAGAAAACCATCTCCAAAGCCAAAGGGCAGCCCCGAGAGCCACAGGTGTACACCCTGCCCCCATCCCAGGAGGAGATGACCAAGAACCAGGTCAGCCTGACCTGCCTGGTCAAAGGCTTCTACCCCAGCGACATCGCCGTGGAGTGGGAGAGCAATGGGCAGCCGGAGAACAACTACAAGACCACGCCTCCCGTGCTGGACTCCGACGGCTCCTTCTTCCTCTACAGCAGGCTAACCGTGGACAAGAGCAGGTGGCAGGAGGGGAATGTCTTCTCATGCTCCGTGATGCATGAGGCTCTGCACAACCACTACACACAGAAGAGCCTCTCCCTGTCTCTGGGTAAA

SEQ ID NO: 70 - protein, 327 aa, Homo Sapien
ASTKGPSVFPLAPCSRSTSESTAALGCLVKDYFPEPVTVSWNSGALTSGVHTFPAVLQSSGLYSLSSVVTVPSSSLGTKTYTCNVDHKPSNTKVDKRVESKYGPPCPSCPAPEFLGGPSVFLFPPKPKDTLMISRTPEVTCVVVDVSQEDPEVQFNWYVDGVEVHNAKTKPREEQFNSTYRVVSVLTVLHQDWLNGKEYKCKVSNKGLPSSIEKTISKAKGQPREPQVYTLPPSQEEMTKNQVSLTCLVKGFYPSDIAVEWESNGQPENNYKTTPPVLDSDGSFFLYSRLTVDKSRWQEGNVFSCSVMHEALHNHYTQKSLSLSLGK

SEQ ID NO: 71 - protein, 981 aa, Homo Sapien
GCTTCCACCAAGGGCCCATCCGTCTTCCCCCTGGCGCCCTGCTCCAGGAGCACCTCCGAGAGCACAGCCGCCCTGGGCTGCCTGGTCAAGGACTACTTCCCCGAACCGGTGACGGTGTCGTGGAACTCAGGCGCCCTGACCAGCGGCGTGCACACCTTCCCGGCTGTCCTACAGTCCTCAGGACTCTACTCCCTCAGCAGCGTGGTGACCGTGCCCTCCAGCAGCTTGGGCACGAAGACCTACACCTGCAACGTAGATCACAAGCCCAGCAACACCAAGGTGGACAAGAGAGTTGAGTCCAAATATGGTCCCCCGTGCCCATCATGCCCAGCACCTGAGTTCCTGGGGGGACCATCAGTCTTCCTGTTCCCCCCAAAACCCAAGGACACTCTCATGATCTCCCGGACCCCTGAGGTCACGTGCGTGGTGGTGGACGTGAGCCAGGAAGACCCCGAGGTCCAGTTCAACTGGTACGTGGATGGCGTGGAGGTGCATAATGCCAAGACAAAGCCGCGGGAGGAGCAGTTCAACAGCACGTACCGTGTGGTCAGCGTCCTCACCGTCGTGCACCAGGACTGGCTGAACGGCAAGGAGTACAAGTGCAAGGTCTCCAACAAAGGCCTCCCGTCCTCCATCGAGAAAACCATCTCCAAAGCCAAAGGGCAGCCCCGAGAGCCACAGGTGTACACCCTGCCCCCATCCCAGGAGGAGATGACCAAGAACCAGGTCAGCCTGACCTGCCTGGTCAAAGGCTTCTACCCCAGCGACATCGCCGTGGAGTGGGAGAGCAATGGGCAGCCGGAGAACAACTACAAGACCACGCCTCCCGTGCTGGACTCCGACGGCTCCTTCTTCCTCTACAGCAGGCTAACCGTGGACAAGAGCAGGTGGCAGGAGGGGAATGTCTTCTCATGCTCCGTGATGCATGAGGCTCTGCACAACCACTACACGCAGAAGAGCCTCTCCCTGTCTCTGGGTAAA

SEQ ID NO: 72 - protein, 327 aa, Homo Sapien
ASTKGPSVFPLAPCSRSTSESTAALGCLVKDYFPEPVTVSWNSGALTSGVHTFPAVLQSSGLYSLSSVVTVPSSSLGTKTYTCNVDHKPSNTKVDKRVESKYGPPCPSCPAPEFLGGPSVFLFPPKPKDTLMISRTPEVTCVVVDVSQEDPEVQFNWYVDGVEVHNAKTKPREEQFNSTYRVVSVLTVVHQDWLNGKEYKCKVSNKGLPSSIEKTISKAKGQPREPQVYTLPPSQEEMTKNQVSLTCLVKGFYPSDIAVEWESNGQPENNYKTTPPVLDSDGSFFLYSRLTVDKSRWQEGNVFSCSVMHEALHNHYTQKSLSLSLGK

SEQ ID NO: 73 - protein, 981 aa, Homo Sapien
GCTTCCACCAAGGGCCCATCCGTCTTCCCCCTGGCGCCCTGCTCCAGGAGCACCTCCGAGAGCACAGCCGCCCTGGGCTGCCTGGTCAAGGACTACTTCCCCGAACCGGTGACGGTGTCGTGGAACTCAGGCGCCCTGACCAGCGGCGTGCACACCTTCCCGGCTGTCCTACAGTCCTCAGGACTCTACTCCCTCAGCAGCGTGGTGACCGTGCCCTCCAGCAGCTTGGGCACGAAGACCTACACCTGCAACGTAGATCACAAGCCCAGCAACACCAAGGTGGACAAGAGAGTTGAGTCCAAATATGGTCCCCCATGCCCATCATGCCCAGCACCTGAGTTCCTGGGGGGACCATCAGTCTTCCTGTTCCCCCCAAAACCCAAGGACACTCTCATGATCTCCCGGACCCCTGAGGTCACGTGCGTGGTGGTGGACGTGAGCCAGGAAGACCCCGAGGTCCAGTTCAACTGGTACGTGGATGGCGTGGAGGTGCATAATGCCAAGACAAAGCCGCGGGAGGAGCAGTTCAACAGCACGTACCGTGTGGTCAGCGTCCTCACCGTCCTGCACCAGGACTGGCTGAACGGCAAGGAGTACAAGTGCAAGGTCTCCAACAAAGGCCTCCCGTCCTCCATCGAGAAAACCATCTCCAAAGCCAAAGGGCAGCCCCGAGAGCCACAGGTGTACACCCTGCCCCCATCCCAGGAGGAGATGACCAAGAACCAGGTCAGCCTGACCTGCCTGGTCAAAGGCTTCTACCCCAGCGACATCGCCGTGGAGTGGGAGAGCAATGGGCAGCCGGAGAACAACTACAAGACCACGCCTCCCGTGCTGGACTCCGACGGCTCCTTCTTCCTCTACAGCAAGCTCACCGTGGACAAGAGCAGGTGGCAGGAGGGGAACGTCTTCTCATGCTCCGTGATGCATGAGGCTCTGCACAACCACTACACGCAGAAGAGCCTCTCCCTGTCTCTGGGTAAA

SEQ ID NO: 74 - protein, 327 aa, Homo Sapien
ASTKGPSVFPLAPCSRSTSESTAALGCLVKDYFPEPVTVSWNSGALTSGVHTFPAVLQSSGLYSLSSVVTVPSSSLGTKTYTCNVDHKPSNTKVDKRVESKYGPPCPSCPAPEFLGGPSVFLFPPKPKDTLMISRTPEVTCVVVDVSQEDPEVQFNWYVDGVEVHNAKTKPREEQFNSTYRVVSVLTVLHQDWLNGKEYKCKVSNKGLPSSIEKTISKAKGQPREPQVYTLPPSQEEMTKNQVSLTCLVKGFYPSDIAVEWESNGQPENNYKTTPPVLDSDGSFFLYSKLTVDKSRWQEGNVFSCSVMHEALHNHYTQKSLSLSLGK

SEQ ID NO: 75 - protein, 981 aa, Homo Sapien
GCCTCCACCAAGGGCCCATCCGTCTTCCCCCTGGCGCCCTGCTCCAGGAGCACCTCCGAGAGCACGGCCGCCCTGGGCTGCCTGGTCAAGGACTACTTCCCCGAACCAGTGACGGTGTCGTGGAACTCAGGCGCCCTGACCAGCGGCGTGCACACCTTCCCGGCTGTCCTACAGTCCTCAGGACTCTACTCCCTCAGCAGCGTGGTGACCGTGCCCTCCAGCAGCTTGGGCACGAAGACCTACACCTGCAACGTAGATCACAAGCCCAGCAACACCAAGGTGGACAAGAGAGTTGAGTCCAAATATGGTCCCCCATGCCCACCATGCCCAGCGCCTGAATTTGAGGGGGGACCATCAGTCTTCCTGTTCCCCCCAAAACCCAAGGACACTCTCATGATCTCCCGGACCCCTGAGGTCACGTGCGTGGTGGTGGACGTGAGCCAGGAAGACCCCGAGGTCCAGTTCAACTGGTACGTGGATGGCGTGGAGGTGCATAATGCCAAGACAAAGCCGCGGGAGGAGCAGTTCAACAGCACGTACCGTGTGGTCAGCGTCCTCACCGTCCTGCACCAGGACTGGCTGAACGGCAAGGAGTACAAGTGCAAGGTCTCCAACAAAGGCCTCCCGTCATCGATCGAGAAAACCATCTCCAAAGCCAAAGGGCAGCCCCGAGAGCCACAGGTGTACACCCTGCCCCCATCCCAGGAGGAGATGACCAAGAACCAGGTCAGCCTGACCTGCCTGGTCAAAGGCTTCTACCCCAGCGACATCGCCGTGGAGTGGGAGAGCAATGGGCAGCCGGAGAACAACTACAAGACCACGCCTCCCGTGCTGGACTCCGACGGATCCTTCTTCCTCTACAGCAGGCTAACCGTGGACAAGAGCAGGTGGCAGGAGGGGAATGTCTTCTCATGCTCCGTGATGCATGAGGCTCTGCACAACCACTACACACAGAAGAGCCTCTCCCTGTCTCTGGGTAAA

SEQ ID NO: 76 - protein, 981 aa, Homo Sapien
GCCTCCACCAAGGGACCTAGCGTGTTCCCTCTCGCCCCCTGTTCCAGGTCCACAAGCGAGTCCACCGCTGCCCTCGGCTGTCTGGTGAAAGACTACTTTCCCGAGCCCGTGACCGTCTCCTGGAATAGCGGAGCCCTGACCTCCGGCGTGCACACATTTCCCGCCGTGCTGCAGAGCAGCGGACTGTATAGCCTGAGCAGCGTGGTGACCGTGCCCAGCTCCAGCCTCGGCACCAAAACCTACACCTGCAACGTGGACCACAAGCCCTCCAACACCAAGGTGGACAAGCGGGTGGAGAGCAAGTACGGCCCCCCTTGCCCTCCTTGTCCTGCCCCTGAGTTCGAGGGAGGACCCTCCGTGTTCCTGTTTCCCCCCAAACCCAAGGACACCCTGATGATCTCCCGGACACCCGAGGTGACCTGTGTGGTCGTGGACGTCAGCCAGGAGGACCCCGAGGTGCAGTTCAACTGGTATGTGGACGGCGTGGAGGTGCACAATGCCAAAACCAAGCCCAGGGAGGAGCAGTTCAATTCCACCTACAGGGTGGTGAGCGTGCTGACCGTCCTGCATCAGGATTGGCTGAACGGCAAGGAGTACAAGTGCAAGGTGTCCAACAAGGGACTGCCCAGCTCCATCGAGAAGACCATCAGCAAGGCTAAGGGCCAGCCGAGGGAGCCCCAGGTGTATACCCTGCCTCCTAGCCAGGAAGAGATGACCAAGAACCAAGTGTCCCTGACCTGCCTGGTGAAGGGATTCTACCCCTCCGACATCGCCGTGGAGTGGGAGAGCAATGGCCAGCCCGAGAACAACTACAAAACAACCCCTCCCGTGCTCGATAGCGACGGCAGCTTCTTTCTCTACAGCCGGCTGACAGTGGACAAGAGCAGGTGGCAGGAGGGCAACGTGTTCTCCTGTTCCGTGATGCACGAGGCCCTGCACAATCACTACACCCAGAAGAGCCTCTCCCTGTCCCTGGGCAAG

SEQ ID NO: 77 - protein, 981 aa, Homo Sapien
GCCAGCACCAAGGGCCCTTCCGTGTTCCCCCTGGCCCCTTGCAGCAGGAGCACCTCCGAATCCACAGCTGCCCTGGGCTGTCTGGTGAAGGACTACTTTCCCGAGCCCGTGACCGTGAGCTGGAACAGCGGCGCTCTGACATCCGGCGTCCACACCTTTCCTGCCGTCCTGCAGTCCTCCGGCCTCTACTCCCTGTCCTCCGTGGTGACCGTGCCTAGCTCCTCCCTCGGCACCAAGACCTACACCTGTAACGTGGACCACAAACCCTCCAACACCAAGGTGGACAAACGGGTCGAGAGCAAGTACGGCCCTCCCTGCCCTCCTTGTCCTGCCCCCGAGTTCGAAGGCGGACCCAGCGTGTTCCTGTTCCCTCCTAAGCCCAAGGACACCCTCATGATCAGCCGGACACCCGAGGTGACCTGCGTGGTGGTGGATGTGAGCCAGGAGGACCCTGAGGTCCAGTTCAACTGGTATGTGGATGGCGTGGAGGTGCACAACGCCAAGACAAAGCCCCGGGAAGAGCAGTTCAACTCCACCTACAGGGTGGTCAGCGTGCTGACCGTGCTGCATCAGGACTGGCTGAACGGCAAGGAGTACAAGTGCAAGGTCAGCAATAAGGGACTGCCCAGCAGCATCGAGAAGACCATCTCCAAGGCTAAAGGCCAGCCCCGGGAACCTCAGGTGTACACCCTGCCTCCCAGCCAGGAGGAGATGACCAAGAACCAGGTGAGCCTGACCTGCCTGGTGAAGGGATTCTACCCTTCCGACATCGCCGTGGAGTGGGAGTCCAACGGCCAGCCCGAGAACAATTATAAGACCACCCCTCCCGTCCTCGACAGCGACGGATCCTTCTTTCTGTACTCCAGGCTGACCGTGGATAAGTCCAGGTGGCAGGAAGGCAACGTGTTCAGCTGCTCCGTGATGCACGAGGCCCTGCACAATCACTACACCCAGAAGTCCCTGAGCCTGTCCCTGGGAAAG

SEQ ID NO: 78 - protein, 327 aa, Homo Sapien
ASTKGPSVFPLAPCSRSTSESTAALGCLVKDYFPEPVTVSWNSGALTSGVHTFPAVLQSSGLYSLSSVVTVPSSSLGTKTYTCNVDHKPSNTKVDKRVESKYGPPCPPCPAPEFEGGPSVFLFPPKPKDTLMISRTPEVTCVVVDVSQEDPEVQFNWYVDGVEVHNAKTKPREEQFNSTYRVVSVLTVLHQDWLNGKEYKCKVSNKGLPSSIEKTISKAKGQPREPQVYTLPPSQEEMTKNQVSLTCLVKGFYPSDIAVEWESNGQPENNYKTTPPVLDSDGSFFLYSRLTVDKSRWQEGNVFSCSVMHEALHNHYTQKSLSLSLGK

SEQ ID NO: 79 - protein, 981 aa, synthetic construct
  REGION 1..981: note = Synthetic Constant Region
GCCTCCACCAAGGGCCCATCCGTCTTCCCCCTGGCGCCCTGCTCCAGGAGCACCTCCGAGAGCACGGCCGCCCTGGGCTGCCTGGTCAAGGACTACTTCCCCGAACCAGTGACGGTGTCGTGGAACTCAGGCGCCCTGACCAGCGGCGTGCACACCTTCCCGGCTGTCCTACAGTCCTCAGGACTCTACTCCCTCAGCAGCGTGGTGACCGTGCCCTCCAGCAGCTTGGGCACGAAGACCTACACCTGCAACGTAGATCACAAGCCCAGCAACACCAAGGTGGACAAGAGAGTTGAGTCCAAATATGGTCCCCCATGCCCACCATGCCCAGCGCCTCCAGTTGCGGGGGGACCATCAGTCTTCCTGTTCCCCCCAAAACCCAAGGACACTCTCATGATCTCCCGGACCCCTGAGGTCACGTGCGTGGTGGTGGACGTGAGCCAGGAAGACCCCGAGGTCCAGTTCAACTGGTACGTGGATGGCGTGGAGGTGCATAATGCCAAGACAAAGCCGCGGGAGGAGCAGTTCAACAGCACGTACCGTGTGGTCAGCGTCCTCACCGTCCTGCACCAGGACTGGCTGAACGGCAAGGAGTACAAGTGCAAGGTCTCCAACAAAGGCCTCCCGTCATCGATCGAGAAAACCATCTCCAAAGCCAAAGGGCAGCCCCGAGAGCCACAGGTGTACACCCTGCCCCCATCCCAGGAGGAGATGACCAAGAACCAGGTCAGCCTGACCTGCCTGGTCAAAGGCTTCTACCCCAGCGACATCGCCGTGGAGTGGGAGAGCAATGGGCAGCCGGAGAACAACTACAAGACCACGCCTCCCGTGCTGGACTCCGACGGATCCTTCTTCCTCTACAGCAGGCTAACCGTGGACAAGAGCAGGTGGCAGGAGGGGAATGTCTTCTCATGCTCCGTGATGCATGAGGCTCTGCACAACCACTACACACAGAAGAGCCTCTCCCTGTCTCTGGGTAAA

SEQ ID NO: 80 - protein, 327 aa, Homo Sapien
ASTKGPSVFPLAPCSRSTSESTAALGCLVKDYFPEPVTVSWNSGALTSGVHTFPAVLQSSGLYSLSSVVTVPSSSLGTKTYTCNVDHKPSNTKVDKRVESKYGPPCPPCPAPPVAGGPSVFLFPPKPKDTLMISRTPEVTCVVVDVSQEDPEVQFNWYVDGVEVHNAKTKPREEQFNSTYRVVSVLTVLHQDWLNGKEYKCKVSNKGLPSSIEKTISKAKGQPREPQVYTLPPSQEEMTKNQVSLTCLVKGFYPSDIAVEWESNGQPENNYKTTPPVLDSDGSFFLYSRLTVDKSRWQEGNVFSCSVMHEALHNHYTQKSLSLSLGK

SEQ ID NO: 81 - protein, 321 aa, Homo Sapien
CGTACGGTGGCCGCTCCCTCCGTGTTCATCTTCCCACCTTCCGACGAGCAGCTGAAGTCCGGCACCGCTTCTGTCGTGTGCCTGCTGAACAACTTCTACCCCCGCGAGGCCAAGGTGCAGTGGAAGGTGGACAACGCCCTGCAGTCCGGCAACTCCCAGGAATCCGTGACCGAGCAGGACTCCAAGGACAGCACCTACTCCCTGTCCTCCACCCTGACCCTGTCCAAGGCCGACTACGAGAAGCACAAGGTGTACGCCTGCGAAGTGACCCACCAGGGCCTGTCTAGCCCCGTGACCAAGTCTTTCAACCGGGGCGAGTGT

SEQ ID NO: 82 - protein, 107 aa, Homo Sapien [sequence omitted]

SEQ ID NO: 83 - protein, 321 aa, Homo Sapien
CGAACTGTGGCTGCACCATCTGTCTTCATCTTCCCGCCATCTGATGAGCAGTTGAAATCTGGAACTGCCTCTGTTGTGTGCCTGCTGAATAACTTCTATCCCAGAGAGGCCAAAGTACAGCGGAAGGTGGATAACGCCCTCCAATCGGGTAACTCCCAGGAGAGTGTCACAGAGCAGGAGAGCAAGGACAGCACCTACAGCCTCAGCAGCACCCTGACGCTGAGCAAAGCAGACTACGAGAAACACAAAGTCTACGCCTGCGAAGTCACCCATCAGGGCCTGAGCTCGCCCGTCACAAAGAGCTTCAACAGGGGAGAGTGT

SEQ ID NO: 84 - protein, 107 aa, Homo Sapien
RTVAAPSVFIFPPSDEQLKSGTASVVCLLNNFYPREAKVQWKVDNALQSGNSQESVTEQESKDSTYSLSSTLTLSKADYEKHKVYAGEVTHQGLSSPVTKSFNRGEC

SEQ ID NO: 85 - protein, 321 aa, Homo Sapien; identical to SEQ ID NO: 83

SEQ ID NO: 86 - protein, 107 aa, Homo Sapien
RTVAAPSVFIFPPSDEQLKSGTASVVCLLNNFYPREAKVQRKVDNALQSGNSQESVTEQESKDSTYSLSSTLTLSKADYEKHKVYACEVTHQGLSSPVTKSFNRGEC

SEQ ID NO: 87 - protein, 321 aa, Homo Sapien
CGAACTGTGGCTGCACCATCTGTCTTCATCTTCCCGCCATCTGATGAGCAGTTGAAATCTGGAACTGCCTCTGTTGTGTGCCTGCTGAATAACTTCTATCCCAGAGAGGCCAAAGTACAGTGGAAGGTGGATAACGCCCTCCAATCGGGTAACTCCCAGGAGAGTGTCACAGAGCAGGACAGCAAGGACAGCACCTACAGCCTCAGCAGCACCCTGACGCTGAGCAAAGCAGACTACGAGAAACACAAACTCTACGCCTGCGAAGTCACCCATCAGGGCCTGAGCTCGCCCGTCACAAAGAGCTTCAACAGGGGAGAGTGT

SEQ ID NO: 88 - protein, 107 aa, Homo Sapien
RTVAAPSVFIFPPSDEQLKSGTASVVCLLNNFYPREAKVQWKVDNALQSGNSQESVTEQDSKDSTYSLSSTLTLSKADYEKHKLYACEVTHQGLSSPVTKSFNRGEC

SEQ ID NO: 89 - protein, 321 aa, Homo Sapien
CGAACTGTGGCTGCACCATCTGTCTTCATCTTCCCGCCATCTGATGAGCAGTTGAAATCTGGAACTGCCTCTGTTGTGTGCCTGCTGAATAACTTCTATCCCAGAGAGGCCAAAGTACAGTGGAAGGTGGATAACGCCCTCCAATCGGGTAACTCCCAGGAGAGTGTCACAGAGCAGGACAGCAAGGACAGCACCTACAGCCTCAGCAACACCCTGACGCTGAGCAAAGCAGACTACGAGAAACACAAAGTCTACGCCTGCGAAGTCACCCATCAGGGCCTGAGCTCGCCCGTCACAAAGAGCTTCAACAGGGGAGAGTGC

SEQ ID NO: 90 - protein, 107 aa, Homo Sapien
RTVAAPSVFIFPPSDEQLKSGTASVVCLLNNFYPREAKVQWKVDNALQSGNSQESVTEQDSKDSTYSLSNTLTLSKADYEKHKVYACEVTHQGLSSPVTKSFNRGEC

SEQ ID NO: 91 - protein, 312 aa, Homo Sapien
CCCAAGGCCAACCCCACGGTCACTCTGTTCCCGCCCTCCTCTGAGGAGCTCCAAGCCAACAAGGCCACACTAGTGTGTCTGATCAGTGACTTCTACCCGGGAGCTGTGACAGTGGCTTGGAAGGCAGATGGCAGCCCCGTCAAGGCGGGAGTGGAGACGACCAAACCCTCCAAACAGAGCAACAACAAGTACGCGGCCAGCAGCTACCTGAGCCTGACGCCCGAGCAGTGGAAGTCCCACAGAAGCTACAGCTGCCAGGTCACGCATGAAGGGAGCACCGTGGAGAAGACAGTGGCCCCTACAGAATGTTCA

SEQ ID NO: 92 - protein, 104 aa, Homo Sapien
PKANPTVTLFPPSSEELQANKATLVCLISDFYPGAVTVAWKADGSPVKAGVETTKPSKQSNNKYAASSYLSLTPEQWKSHRSYSCQVTHEGSTVEKTVAPTECS

SEQ ID NO: 93 - protein, 318 aa, Homo Sapien
GGTCAGCCCAAGGCCAACCCCACTGTCACTCTGTTCCCGCCCTCCTCTGAGGAGCTCCAAGCCAACAAGGCCACACTAGTGTGTCTGATCAGTGACTTCTACCCGGGAGCTGTGACAGTGGCCTGGAAGGCAGATGGCAGCCCCGTCAAGGCGGGAGTGGAGACCACCAAACCCTCCAAACAGAGCAACAACAAGTACGCGGCCAGCAGCTACCTGAGCCTGACGCCCGAGCAGTGGAAGTCCCACAGAAGCTACAGCTGCCAGGTCACGCATGAAGGGAGCACCGTGGAGAAGACAGTGGCCCCTACAGAATGTTCA

SEQ ID NO: 94 - protein, 318 aa, Homo Sapien; identical to SEQ ID NO: 93

SEQ ID NO: 95 - protein, 106 aa, Homo Sapien
GQPKANPTVTLFPPSSEELQANKATLVCLISDFYPGAVTVAWKADGSPVKAGVETTKPSKQSNNKYAASSYLSLTPEQWKSHRSYSCQVTHEGSTVEKTVAPTECS

SEQ ID NO: 96 - protein, 318 aa, Homo Sapien
GGCCAGCCTAAGGCCGCTCCTTCTGTGACCCTGTTCCCCCCATCCTCCGAGGAACTGCAGGCTAACAAGGCCACCCTCGTGTGCCTGATCAGCGACTTCTACCCTGGCGCCGTGACCGTGGCCTGGAAGGCTGATAGCTCTCCTGTGAAGGCCGGCGTGGAAACCACCACCCCTTCCAAGCAGTCCAACAACAAATACGCCGCCTCCTCCTACCTGTCCCTGACCCCTGAGCAGTGGAAGTCCCACCGGTCCTACAGCTGCCAAGTGACCCACGAGGGCTCCACCGTGGAAAAGACCGTGGCTCCTACCGAGTGCTCC

SEQ ID NO: 97 - protein, 318 aa, Homo Sapien
GGCCAGCCTAAAGCTGCCCCCAGCGTCACCCTGTTTCCTCCCTCCAGCGAGGAGCTCCAGGCCAACAAGGCCACCCTCGTGTGCCTGATCTCCGACTTCTATCCCGGCGCTGTGACCGTGGCTTGGAAAGCCGACTCCAGCCCTGTCAAAGCCGGCGTGGAGACCACCACACCCTCCAAGCAGTCCAACAACAAGTACGCCGCCTCCAGCTATCTCTCCCTGACCCCTGAGCAGTGGAAGTCCCACCGGTCCTACTCCTGTCAGGTGACCCACGAGGGCTCCACCGTGGAAAAGACCGTCGCCCCCACCGAGTGCTCC

SEQ ID NO: 98 - protein, 106 aa, Homo Sapien
GQPKAAPSVTLFPPSSEELQANKATLVCLISDFYPGAVTVAWKADSSPVKAGVETTTPSKQSNNKYAASSYLSLTPEQWKSHRSYSCQVTHEGSTVEKTVAPTECS

SEQ ID NO: 99 - protein, 318 aa, Homo Sapien
GGTCAGCCCAAGGCTGCCCCCTCGGTCACTCTGTTCCCGCCCTCCTCTGAGGAGCTTCAAGCCAACAAGGCCACACTGGTGTGTCTCATAAGTGACTTCTACCCGGGAGCCGTGACAGTGGCCTGGAAGGCAGATAGCAGCCCCGTCAAGGCGGGAGTGGAGACCACCACACCCTCCAAACAAAGCAACAACAAGTACGCGGCCAGCAGCTATCTGAGCCTGACGCCTGAGCAGTGGAAGTCCCACAGAAGCTACAGCTGCCAGGTCACGCATGAAGGGAGCACCGTGGAGAAGACAGTGGCCCCTACAGAATGTTCA

SEQ ID NO: 100 - protein, 106 aa, Homo Sapien; identical to SEQ ID NO: 98

SEQ ID NO: 101 - protein, 312 aa, Homo Sapien
CCCAAGGCTGCCCCCTCGGTCACTCTGTTCCCACCCTCCTCTGAGGAGCTTCAAGCCAACAAGGCCACACTGGTGTGTCTCATAAGTGACTTCTACCCGGGAGCCGTGACAGTTGCCTGGAAGGCAGATAGCAGCCCCGTCAAGGCGGGGGTGGAGACCACCACACCCTCCAAACAAAGCAACAACAAGTACGCGGCCAGCAGCTACCTGAGCCTGACGCCTGAGCAGTGGAAGTCCCACAAAAGCTACAGCTGCCAGGTCACGCATGAAGGGAGCACCGTGGAGAAGACAGTTGCCCCTACGGAATGTTCA

SEQ ID NO: 102 - protein, 104 aa, Homo Sapien
PKAAPSVTLFPPSSEELQANKATLVCLISDFYPGAVTVAWKADSSPVKAGVETTTPSKQSNNKYAASSYLSLTPEQWKSHKSYSCQVTHEGSTVEKTVAPTECS

SEQ ID NO: 103 - protein, 318 aa, Homo Sapien
GGTCAGCCCAAGGCTGCCCCCTCGGTCACTCTGTTCCCACCCTCCTCTGAGGAGCTTCAAGCCAACAAGGCCACACTGGTGTGTCTCATAAGTGACTTCTACCCGGGGCCAGTGACAGTTGCCTGGAAGGCAGATAGCAGCCCCGTCAAGGCGGGGGTGGAGACCACCACACCCTCCAAACAAAGCAACAACAAGTACGCGGCCAGCAGCTACCTGAGCCTGACGCCTGAGCAGTGGAAGTCCCACAAAAGCTACAGCTGCCAGGTCACGCATGAAGGGAGCACCGTGGAGAAGACAGTGGCCCCTACGGAATGTTCA

SEQ ID NO: 104 - protein, 106 aa, Homo Sapien
GQPKAAPSVTLFPPSSEELQANKATLVCLISDFYPGPVTVAWKADSSPVKAGVETTTPSKQSNNKYAASSYLSLTPEQWKSHKSYSCQVTHEGSTVEKTVAPTECS

SEQ ID NO: 105 - protein, 318 aa, Homo Sapien
GGTCAGCCCAAGGCTGCCCCCTCGGTCACTCTGTTCCCACCCTCCTCTGAGGAGCTTCAAGCCAACAAGGCCACACTGGTGTGTCTCATAAGTGACTTCTACCCGGGAGCCGTGACAGTGGCCTGGAAGGCAGATAGCAGCCCCGTCAAGGCGGGAGTGGAGACCACCACACCCTCCAAACAAAGCAACAACAAGTACGCGGCCAGCAGCTACCTGAGCCTGACGCCTGAGCAGTGGAAGTCCCACAAAAGCTACAGCTGCCAGGTCACGCATGAAGGGAGCACCGTGGAGAAGACAGTGGCCCCTACAGAATGTTCA

SEQ ID NO: 106 - protein, 106 aa, Homo Sapien; identical to SEQ ID NO: 98

SEQ ID NO: 107 - protein, 318 aa, Homo Sapien
GGTCAGCCCAAGGCTGCCCCCTCGGTCACTCTGTTCCCGCCCTCCTCTGAGGAGCTTCAAGCCAACAAGGCCACACTGGTGTGTCTCATAAGTGACTTCTACCCGGGAGCCGTGACAGTGGCCTGGAAGGCAGATAGCAGCCCCGTCAAGGCGGGAGTGGAGACCACCACACCCTCCAAACAAAGCAACAACAAGTACGCGGCCAGCAGCTACCTGAGCCTGACGCCTGAGCAGTGGAAGTCCCACAGAAGCTACAGCTGCCAGGTCACGCATGAAGGGAGCACCGTGGAGAAGACAGTGGCCCCTACAGAATGTTCA

SEQ ID NO: 108 - protein, 106 aa, Homo Sapien; identical to SEQ ID NO: 98

SEQ ID NO: 109 - protein, 318 aa, Homo Sapien
GGTCAGCCCAAGGCTGCCCCATCGGTCACTCTGTTCCCGCCCTCCTCTGAGGAGCTTCAAGCCAACAAGGCCACACTGGTGTGCCTGATCAGTGACTTCTACCCGGGAGCTGTGAAAGTGGCCTGGAAGGCAGATGGCAGCCCCGTCAACACGGGAGTGGAGACCACCACACCCTCCAAACAGAGCAACAACAAGTACGCGGCCAGCAGCTACCTGAGCCTGACGCCTGAGCAGTGGAAGTCCCACAGAAGCTACAGCTGCCAGGTCACGCATGAAGGGAGCACCGTGGAGAAGACAGTGGCCCCTGCAGAATGTTCA

SEQ ID NO: 110 - protein, 106 aa, Homo Sapien
GQPKAAPSVTLFPPSSEELQANKATLVCLISDFYPGAVKVAWKADGSPVNTGVETTTPSKQSNNKYAASSYLSLTPEQWKSHRSYSCQVTHEGSTVEKTVAPAECS

SEQ ID NO: 111 - protein, 318 aa, Homo Sapien
GGTCAGCCCAAGGCTGCCCCATCGGTCACTCTGTTCCCACCCTCCTCTGAGGAGCTTCAAGCCAACAAGGCCACACTGGTGTGTCTCGTAAGTGACTTCTACCCGGGAGCCGTGACAGTGGCCTGGAAGGCAGATGGCAGCCCCGTCAAGGTGGGAGTGGAGACCACCAAACCCTCCAAACAAAGCAACAACAAGTATGCGGCCAGCAGCTACCTGAGCCTGACGCCCGAGCAGTGGAAGTCCCACAGAAGCTACAGCTGCCGGGTCACGCATGAAGGGAGCACCGTGGAGAAGACAGTGGCCCCTGCAGAATGCTCT

SEQ ID NO: 112 - protein, 106 aa, Homo Sapien
GQPKAAPSVTLFPPSSEELQANKATLVCLVSDFYPGAVTVAWKADGSPVKVGVETTKPSKQSNNKYAASSYLSLTPEQWKSHRSYSCRVTHEGSTVEKTVAPAECS

SEQ ID NO: 113 - protein, 318 aa, Homo Sapien
GGTCAGCCCAAGGCTGCCCCCTCGGTCACTCTGTTCCCACCCTCCTCTGAGGAGCTTCAAGCCAACAAGGCCACACTGGTGTGTCTCGTAAGTGACTTCAACCCGGGAGCCGTGACAGTGGCCTGGAAGGCAGATGGCAGCCCCGTCAAGGTGGGAGTGGAGACCACCAAACCCTCCAAACAAAGCAACAACAAGTATGCGGCCAGCAGCTACCTGAGCCTGACGCCCGAGCAGTGGAAGTCCCACAGAAGCTACAGCTGCCGGGTCACGCATGAAGGGAGCACCGTGGAGAAGACAGTGGCCCCTGCAGAATGCTCT

SEQ ID NO: 114 - protein, 106 aa, Homo Sapien
GQPKAAPSVTLFPPSSEELQANKATLVCLVSDFNPGAVTVAWKADGSPVKVGVETTKPSKQSNNKYAASSYLSLTPEQWKSHRSYSCRVTHEGSTVEKTVAPAECS